European Patent Application EP 4 585 049 A2, published July 16, 2025. Title: Eicosapentaenoic Acid-Producing Microorganisms, Fatty Acid Compositions, and Methods of Making and Uses Thereof. Applicant: Pfeifer III, Joseph W. Application undefined To be assigned, filed July 20, 2012. The sequence listing filed with the application follows.

SEQUENCE LISTING (2 sequences)

SEQ ID NO: 1 - DNA, 1705 bp, Thraustochytrium sp.
  source 1..1705: mol_type = genomic DNA
aagatacctggttgatcctgccagtagtcatacgctcgtctcaaagattaagccatgcatgtgtcagtataaatacttttactttgaaactgcgaacggctcattaaatcagtaattatctacatggtaacgaaaattatatggataaccgtagtaattctagggctaatacatgcgtaaaatctgggtaactggatgcatttattggattgaagccaacattaaaaggtgattcacgataactaagcggagcgttttaggacgctgaatcattcgagtttctgccctatcagctgtcgatggtaaggtattggcttaccatggcgttaacgggtaacggagaattagggttcgattccggagagggagcctgagagacggctaccacatccaaggaaggcagcaggcgcgtaaattgcccaatgagaacttctcgaggcagtgacaagaaatatcaaagtgatgccgttaggtattgcatttgaaatgagaacgatgtacaacttctaacgatgatcaattggagggcaagtctggtgccagcagccgcggtaattccagctccaatagcgtatactaacgttgctgcagttaaaacgcccgtagttgaattagtatcatggtattttaaccttattcgatgaatttgagttgaaagctaggatatataggaagcgattcctcatttactgtaaaaaaattagagtgtttcacacagatcgtaagatcgggatatattagtatggaataataagataggactttggtgctattttgttggtttgcacaccaaagtaatgattaatagggacagttgggggtattcgtatttaattgtcagaggtgaaattcttggatttatgaaagacgaactactgcgaaagcatttaccaaggatgttttcattaatcaaggacgaaagttaggggatcgaagatgattagataccatcgtagtcttaaccataaactatgccgactgaggattcttgaaatttgtaaatgaatttaagagcactccatgagaaatcaaagtctttgggttccggggggagtatggtcgcaagtctgaaacttaaaggaattgacggaagggcaccaccaggagtggagcctgcggcttaatttgactcaacacgggaaaacttaccaggtccagacatagtgaggattgacagattgatagctctttcttgattctatgggtggtggtgcatggccgttcttagttggtggtttgaactgtctgcttaattgcgttaacgaacgagacctcagcctactaaatagtatgttgtttagtaataaatgatatgacttcttagagggacatttcgggtttaccggaaggaagtttgaggcaataacaggtctgtgatgcccttagatgttctgggccgcacgcgcgctacactgacgagctcaacaagtaatatttggttgtctggaaggattgcctaatcttttaaatactcgtcgtgatggggctagattcttgtaattattaatctccaacgaggaattcctagtaaacgcaagtcatcagcttgcattgattacgtccctgccctttgtacacaccgcccgtcgcacctaccgattggatggtccggtgaaatcttcggatgtttttttacaatagtagagagacaaaagttgagtaaaccttaccatctagaggaaggtgaagtcgtaacaaggatctt

SEQ ID NO: 2 - DNA, 1713 bp, Schizochytrium sp.
  source 1..1713: mol_type = genomic DNA
acctggttgatcctgccagctgtcatttgctcgtctaaaagattaagccatgcatgtctaagtataaacaaattatacggtgaaactgcgaacggctcattatatcagttatagtttctttgatagtgtatttctatatctatttggataactgtggcaattctagagctaacacatgctttcgagtgggactttttggtaccactgcatttattagattttgaagccaacgtaaaattggtgattcatgataactttgcgaatcgcagtagcgtcttgtacgcggcgatgaatcattcaagtttctgccccatcagctgtcgatggtacggtattggcctaccatggctttcacgggtgacggagaattagggtttgattccggagaggacgcttgagagacggcgaccacatccaaggaaggcagcaggcgcgtaaattacccaatggggactccccgaggtagtgacaagaaataaaaatgaggagcgctttgcgtttttcaatttgaatgagagaatcgtacaatcctcatcgaggatcaattggagggcaagtctggtgccagcagccgcggtaactccagctccaatagcaaatattagagttgttgcagttaaaaagctcgtagttgaatttccgatagtctttggccgtgtccttggtctcgtatcatgggtttattgtgccaagatgatcgtcctctatggttagtgatagtcatagtcgtttactgtaaaaaaactggagtgtttaaagcatttctttgggaaaggtacatattagtataggataattagataggacctgtgattcttatttggttggtttgtgagtcatggtaatgattaatagggacaatcgggggtattcgaatttaattgtcagaggtgaaattcttggatttaagaaagtcgaactactgcgaaggcatttaccaaggatgttttcattaataaagaacgaaagttaggggatcgaagatgattagataccatcgtagtcttaactgtaaactatgccgacttgcgattgtccgtcgttgttttttcaaaaaagagacctgggcagcagcacatgagaaatcaaagtttttgggttccggggggagtatggtcgcaaggctgaaacttaaaggaattgacggaagggcaccaccaggagtggagcctgcggcttaattcgactcaacacgggaaaacttaccaggtccagacatagtaaggattgacagattgagagctctttcttgattctatgggtggtggtgcatggccgttcttagttggtggagtgatttgtctggttaattccgttaacgaacgagacctcagcctactaaatagtggtgcatattgtgagatatgtgacaaaaatcgcttcttagagggacatttcgggtttaccggaaggaagtttgaggcaataacaggtctgtgatgcccctagatgttctgggccgcacgcgcgctacaatgacagattcaacaagtccggtagtggagcttttgcttctctattattacttttccgagaggaatggttaatcttctaaatgtctgtcgtgatggggctagatttttgcaattattaatctccaacgaggaattcctagtaaacgcaagtcatcagcttgcattgattacgtccctgccctttgtacacaccgcccgtcgcacctaccgattgaacggtcctatgaaatcttcggat